European Patent Specification EP 3 782 653 B1, published March 19, 2025. Title: COMPOSITION COMPRISING PEGYLATED ARGININE DEIMINASE. Applicant: POLARIS GROUP. The sequence listing filed with the application follows.

SEQUENCE LISTING (4 sequences)

SEQ ID NO: 1 - protein, 409 aa, Mycoplasma hominis
MSVFDSKFNGIHVYSEIGELETVLVHEPGREIDYITPARLDELLFSAILESHDARKEHQSFVKIMKDRGINVVELTDLVAETYDLASKAAKEEFIETFLEETVPVLTEANKKAVRAFLLSKPTHEMVEFMMSGITKYELGVESENELIVDPMPNLYFTRDPFASVGNGVTIHFMRYIVRRRETLFARFVFRNHPKLVKTPWYYDPAMKMPIEGGDVFIYNNETLVVGVSERTDLDTITLLAKNIKANKEVEFKRIVAINVPKWTNLMHLDTWLTMLDKNKFLYSPIANDVFKFWDYDLVNGGAEPQPQLNGLPLDKLLASIINKEPVLIPIGGAGATEMEIARETNFDGTNYLAIKPGLVIGYDRNEKTNAALKAAGITVLPFHGNQLSLGMGNARCMSMPLSRKDVKW

SEQ ID NO: 2 - protein, 409 aa, Mycoplasma hominis
MSVFDSKFNGIHVYSEIGELETVLVHEPGREIDYITPARLDELLFSAILESHDARKEHQSFVKIMKDRGINVVELTDLVAETYDLASKAAKEEFIETFLEETVPVLTEANKEAVRAFLLSKPTHEMVEFMMSGITKYELGVESENELIVDPMPNLYFTRDPFASVGNGVTIHFMRYIVRRRETLFARFVFRNHPKLVKTPWYYDPAMKMSIEGGDVFIYNNETLVVGVSERTDLDTITLLAKNIKANKEVEFKRIVAINVPKWTNLMHLDTWLTMLDKNKFLYSPIANDVFKFWDYDLVNGGAEPQPQLNGLPLDKLLASIINKEPVLIPIGGAGATEMEIARETNFDGTNYLAIKPGLVIGYDRNEKTNAALKAAGITVLPFHGNQLSLGMGNARCMSMPLSRKDVKW

SEQ ID NO: 3 - DNA, 18 bp, Homo sapiens
  misc_feature (1)..(18): Forward PCR primer used to amplify argininosuccinate synthetase cDNA
tttaagcagactaagggg

SEQ ID NO: 4 - DNA, 21 bp, Homo sapiens
  misc_feature (1)..(21): Reverse PCR primer used to amplify argininosuccinate synthetase cDNA
ccatcccaggttataagcaca